European Patent Specification EP 3 659 147 B1, published November 5, 2025. Title: DNA-BASED DATA STORAGE AND RETRIEVAL. Applicant: Nanjing GenScript Biotech Co., Ltd. Application EP18838636.1. The sequence listing filed with the application follows.

SEQUENCE LISTING (415 sequences)

SEQ ID NO: 1 - DNA, 87 bp, Artificial Sequence
  Synthetic Construct
ttccctaatagtggagtcgagtagagaaactgactccctgaggacacatcatgcgctcgacgtccatgttgacgtgtgtctcctcag

SEQ ID NO: 2 - DNA, 87 bp, Artificial Sequence
  Synthetic Construct
ttcctacgagagtacgtgtcttattacgcatcatctttcgtcacttacggtttagtccagcgaactgagcgattccgtagagctcga

SEQ ID NO: 3 - DNA, 87 bp, Artificial Sequence
  Synthetic Construct
ttcctgatcttcgagcgagcggacttcgagttaacgttgtatctacgtctgtctggacctgtcagacgactgttgcagtgtcgtcct

SEQ ID NO: 4 - DNA, 87 bp, Artificial Sequence
  Synthetic Construct
ttcctgatgtagcacagcatcgatgtgtacggatagttgatctcagagtgacctaatgagtcgggagtcccaccaatcatccagcga

SEQ ID NO: 5 - DNA, 87 bp, Artificial Sequence
  Synthetic Construct
ttcctaacttcgagtggagcgatgtatggagctcctagattctcaacaccaaatgtactaactactctagtcttatgtataaaccac

SEQ ID NO: 6 - DNA, 87 bp, Artificial Sequence
  Synthetic Construct
ttctacgctcgttgcaatcgattctctgtcatatatcgcactatcctagacagtctcgctgctacaccgtgagatgtggtctgaact

SEQ ID NO: 7 - DNA, 87 bp, Artificial Sequence
  Synthetic Construct
ttcctgcacgagagatctgtgggtcatatgcagtagatggattgctgtgtctctccagcttctgctgagctgtgttagtgtttcgga

SEQ ID NO: 8 - DNA, 87 bp, Artificial Sequence
  Synthetic Construct
ttcctacagagactaagtactccaatcggaatcgtccgagctggacgcttctgtatcatagtcaagacgcagaatatagaccatgag

SEQ ID NO: 9 - DNA, 87 bp, Artificial Sequence
  Synthetic Construct
ttcctacgcatcgagtagtcagtcagcgagagatctactactcataagggtcctgtctagcaggtcgactctataaatatgccgagt

SEQ ID NO: 10 - DNA, 87 bp, Artificial Sequence
  Synthetic Construct
ttcttgtgcgcaactttgttacgacgcgtggagccttactcatgaataaatcgaggtgtgtagcactcttacgcggtagctcgaagc

SEQ ID NO: 11 - DNA, 87 bp, Artificial Sequence
  Synthetic Construct
ttcctgacaaagaatccgaactctggagtactagtggagaacacgctctattagcgcctacaggctaacttggcgtctgtagcttct

SEQ ID NO: 12 - DNA, 87 bp, Artificial Sequence
  Synthetic Construct
ttcctgaatcgtgcttgtgtcacatcttcaatcgtcagccgagctccttgtagtacacctcctgtcttccgatgttcgcacagcact

SEQ ID NO: 13 - DNA, 87 bp, Artificial Sequence
  Synthetic Construct
ttcttgtagactggtgatactatccataaggattgccctcctcagggattaagaggattacgtacttgaatagtcgtcgtgcgcgga

SEQ ID NO: 14 - DNA, 87 bp, Artificial Sequence
  Synthetic Construct
ttcctcgtcctcctacctgtacgagaggctgagtcttaggattgtgagtacggtagcgctcactgttgacgtagtgtgtcagtccat

SEQ ID NO: 15 - DNA, 87 bp, Artificial Sequence
  Synthetic Construct
ttctgacatcctacttgaagtatctgatgaatcgcgggtggctgagtggatggcggcaaggtgacgactatagctatgttctctcgt

SEQ ID NO: 16 - DNA, 87 bp, Artificial Sequence
  Synthetic Construct
ttcctcccaggctgtgcattcgctatcactatcgcttcacgaagaggtcgcacaacaacggatccgacgggtggtgagggacagctc

SEQ ID NO: 17 - DNA, 87 bp, Artificial Sequence
  Synthetic Construct
ttctgaccttcaggcagttatagacgcgcgtcactcccgttaggcgagtatatcagaacgacacgacctactagaagacatcgatct

SEQ ID NO: 18 - DNA, 87 bp, Artificial Sequence
  Synthetic Construct
ttctgactatctagatgacctagaggagagaagatgcgcttgtagacggctgcgcctaacctccctgcgactgcgagtaagactgtg

SEQ ID NO: 19 - DNA, 87 bp, Artificial Sequence
  Synthetic Construct
ttctgactcatggtatagtagggtcatgcgcagcctccatattcgttgtaggtctgtcgtcagagaaaccgcttcatgagatatcag

SEQ ID NO: 20 - DNA, 87 bp, Artificial Sequence
  Synthetic Construct
ttctgatgagcgggctcttgaggagatttcctccgatagaatgcacgaggatagctaatccagctcagagactcgacagctttcccg

SEQ ID NO: 21 - DNA, 87 bp, Artificial Sequence
  Synthetic Construct
ttctgatgcgcaatcagcatcctcgcgggatcaagcacggatgacgctagagacgtctcgagcttctatacactcctgcgattcttc

SEQ ID NO: 22 - DNA, 87 bp, Artificial Sequence
  Synthetic Construct
ttctgatagcacgcagcaagatcgagagtctcatgtgagatcacttgaggtcctcctatcacaactccacatttgatcggacctcgt

SEQ ID NO: 23 - DNA, 87 bp, Artificial Sequence
  Synthetic Construct
ttctgatatatagtaacacatagcagcaacaagacgcagtctcctctaacgagttgtagaaagcctcctggatgaccggcaagatcg

SEQ ID NO: 24 - DNA, 87 bp, Artificial Sequence
  Synthetic Construct
ttctgatcatcaagtcgtgaggtatctatgccgacggtcggacagatgtgtagtatcaaggtccgagcttacaagctcgtctatctc

SEQ ID NO: 25 - DNA, 87 bp, Artificial Sequence
  Synthetic Construct
ttccctgctctactcggccgtcctggtcgaatggtctcgaagggatattgcttccctcaggatagagcacagcctatgggaagacat

SEQ ID NO: 26 - DNA, 87 bp, Artificial Sequence
  Synthetic Construct
ttccctgtgcgaacttgttgaccgctcgtctgagtcagcgtaggagctctctacttgcactctgagggctacccattggtgcgaaag

SEQ ID NO: 27 - DNA, 87 bp, Artificial Sequence
  Synthetic Construct
ttccctgatctagaggctcctcgattcgacgaggctctcctccctcgtagtatagctgtgatcactacttctaatctgttctgaatg

SEQ ID NO: 28 - DNA, 87 bp, Artificial Sequence
  Synthetic Construct
ttctgattattactccgttgcagcgtctcgctgcgcactgatctctctaacctatgtgcttcaagagactagagcccggtagagcca

SEQ ID NO: 29 - DNA, 87 bp, Artificial Sequence
  Synthetic Construct
ttccctagcatcaaccctctggagggcttaaagtatgctctgactactctgctccgaatcactcgcgatctccgtctcgtgactata

SEQ ID NO: 30 - DNA, 87 bp, Artificial Sequence
  Synthetic Construct
ttccctaagaatctccgaaagctctattctgtaatgccgtctggcaatctggtagacctcttgcagttgttggtcatcctgactaga

SEQ ID NO: 31 - DNA, 87 bp, Artificial Sequence
  Synthetic Construct
ttccctgtcgaggcataggtaatggtatcatctcgcgacatgtagttcgtcaatatcccgccgttcggagcgttaatgatgttctga

SEQ ID NO: 32 - DNA, 87 bp, Artificial Sequence
  Synthetic Construct
ttccctagacagttcccatcatcaacttatagcacaggagtccagtctctcgtcttctgcttcccgcagagtacgatctagtcactc

SEQ ID NO: 33 - DNA, 87 bp, Artificial Sequence
  Synthetic Construct
ttcccggcttaggtgacgcgcatcggatgtactacttgtttaccaccaagcgatggactgacagctcaccgtagtatcgactgatag

SEQ ID NO: 34 - DNA, 87 bp, Artificial Sequence
  Synthetic Construct
ttctatttctaggcgtaggtagtatcacagggtcagaacgtctagtctactgagagaactggattgccacatcgcaatggccgaatc

SEQ ID NO: 35 - DNA, 87 bp, Artificial Sequence
  Synthetic Construct
ttcccagtcttcttatcttcatactagtgttgactcctacctccgcaccagcgtcgaatcatgactacaaataagccatagggttct

SEQ ID NO: 36 - DNA, 87 bp, Artificial Sequence
  Synthetic Construct
ttcccagtaatgatcgtagctgattgatgttaggaccgtatcttgtcttgaccggcgagtcgagacgcagagatctgatgtactagc

SEQ ID NO: 37 - DNA, 87 bp, Artificial Sequence
  Synthetic Construct
ttccctggccgaatctctgtcgtaagaaagctgtgccctgctgtatcgaagagaggcacaagctcaataaagatagagctgtcgtga

SEQ ID NO: 38 - DNA, 87 bp, Artificial Sequence
  Synthetic Construct
ttccctgagtgatgaaagacattatcacgaactccgatcggcgtaccaaagccttgatgcatgtcgccacaggactgcctcgatttc

SEQ ID NO: 39 - DNA, 87 bp, Artificial Sequence
  Synthetic Construct
ttcccaaacttgcaggagtagatcttctgcatagaggtgctgagacgattcggcgcattatgatctgtcgtgaaggctatcgcgagt

SEQ ID NO: 40 - DNA, 87 bp, Artificial Sequence
  Synthetic Construct
ttctatttgtcatgtagcctcgtggcttcgggtggacataactcaggatcagcttctgagtcgttgctggtcactcgacacttgcat

SEQ ID NO: 41 - DNA, 87 bp, Artificial Sequence
  Synthetic Construct
ttctgcagaactcgccgattaacatcttagtcacatgaggatctcgtcggccagcctcgatctgcacgacgatacctgcctccaaga

SEQ ID NO: 42 - DNA, 87 bp, Artificial Sequence
  Synthetic Construct
ttctgcagcatgttctagatcatctatatcaagggaacagtgaatgcaatcccagagccggtcggtcacgacgtccgcccgacaatg

SEQ ID NO: 43 - DNA, 87 bp, Artificial Sequence
  Synthetic Construct
ttcctcggtaagctctctgagggcgagagatgactcgctgtcggcagtcagtagcagccgggcctcttctgctcagtaggcttatta

SEQ ID NO: 44 - DNA, 87 bp, Artificial Sequence
  Synthetic Construct
ttctgccgatgaccgccaacaatgtagagaatgggaccacgcccgctgccaataggaaatagttatagtcatatcatggtgcgatta

SEQ ID NO: 45 - DNA, 87 bp, Artificial Sequence
  Synthetic Construct
ttctgtcgttgaggagattcgaacagagacagtcctctgtgctacatgagacagctactcgagacatgagcgatatagccttactct

SEQ ID NO: 46 - DNA, 87 bp, Artificial Sequence
  Synthetic Construct
ttctgtataccatacacagcgttcgaggtcccttattagctgcgaggaggacatctactaaagctcactcgacattcaaatcgccct

SEQ ID NO: 47 - DNA, 87 bp, Artificial Sequence
  Synthetic Construct
ttctgcatcccacgattggctgcttcgaatcactctctctcagctttacgatgtcgaccttacccttctcatccgatggctgagccg

SEQ ID NO: 48 - DNA, 87 bp, Artificial Sequence
  Synthetic Construct
ttctgcacaactctccgaacaggcggcgctgagcctccatgagtatctgagccttatactaagtctgctcatgcgtgttctagatta

SEQ ID NO: 49 - DNA, 87 bp, Artificial Sequence
  Synthetic Construct
ttctgtactgtgataggttcttagacgatgcagtacactttcctcctactaagacatacaagtagatattagggtggatagtctaat

SEQ ID NO: 50 - DNA, 87 bp, Artificial Sequence
  Synthetic Construct
ttctgcaagtctggaagtcatccgggccgactccacacatgacgacctttccgaacttgtccggacgtcagcgtcctctatttccat

SEQ ID NO: 51 - DNA, 87 bp, Artificial Sequence
  Synthetic Construct
ttctgcaacatgccgtctctacgatcaaaccctggaggatacgtcgagcatttcatactctgtagtccgtctgcggcgatcacgctg

SEQ ID NO: 52 - DNA, 87 bp, Artificial Sequence
  Synthetic Construct
ttcctgttctctaagagaggaccggcgttatgtttcttccgatctttcttcctcccagtgagagtcttcggagtctagagcatgtag

SEQ ID NO: 53 - DNA, 87 bp, Artificial Sequence
  Synthetic Construct
ttctattagccattaaacagagagcgatgctcacagaatgcgtgcctctctggccgattatagtcgatctattcactgcatagcatg

SEQ ID NO: 54 - DNA, 87 bp, Artificial Sequence
  Synthetic Construct
ttcctgccactacacaagtagtctccttctctgccgttggtctctccgcgcagagacgcattctagcatgctccgcagaatgtgagt

SEQ ID NO: 55 - DNA, 87 bp, Artificial Sequence
  Synthetic Construct
ttcccggacgtcagaggccgaggctgctgtgacggcaatgcgcctgacatacctctatcattcgctgtacgagacttccgttatagt

SEQ ID NO: 56 - DNA, 87 bp, Artificial Sequence
  Synthetic Construct
ttcttctcgatctcaaagcagcagggcatcgataagatccgatgatactgcgtctctgagtgagtccctgcacgccaggagtctgcg

SEQ ID NO: 57 - DNA, 87 bp, Artificial Sequence
  Synthetic Construct
ttcctcgctctagagcgtactgctcacccagtataggcttcagagacaggtgtgctcctgactgagcgatgctaggagcgaagccgc

SEQ ID NO: 58 - DNA, 87 bp, Artificial Sequence
  Synthetic Construct
ttctacctctgtggaagcatagatgtctaggacactgcgttagactattcatagggtagacgaatcaaggtgtatgacactagattc

SEQ ID NO: 59 - DNA, 87 bp, Artificial Sequence
  Synthetic Construct
ttctacctaaacgctataggagtcatgcgaagttacgagagaatcaacgataatctcgctatccgtggccgcgtcagaactggcgga

SEQ ID NO: 60 - DNA, 87 bp, Artificial Sequence
  Synthetic Construct
ttctactgtcgaatcatgctcagaccgttggcacgagctgctctaacgcctttctgctagcatagtacgcacacgttattactcttc

SEQ ID NO: 61 - DNA, 87 bp, Artificial Sequence
  Synthetic Construct
ttctattgaaagcctcgaatcgctcgtttagtaacagaggcttcgggattcaagcacaaccctccgtcagagacgccgacatgccct

SEQ ID NO: 62 - DNA, 87 bp, Artificial Sequence
  Synthetic Construct
ttctaccacctacactgccgacgttacagaccgatcttccacactcgaggacaggagatcggcgctgctgatgtgtcgttagatgag

SEQ ID NO: 63 - DNA, 87 bp, Artificial Sequence
  Synthetic Construct
ttctatcagctgagcctcacaaagtagcagaacctcagaggagcgactcagcgcatctcgccattgctgcctcctatccattagatc

SEQ ID NO: 64 - DNA, 87 bp, Artificial Sequence
  Synthetic Construct
ttctatcctttcccactcatgctcttaacgcctgcatctcagacattccaggtgaatccgtgattatagaatacggtctgaccacct

SEQ ID NO: 65 - DNA, 87 bp, Artificial Sequence
  Synthetic Construct
ttctatccactgctcctcactcagcctaagtatcacgcttcaactctcacagtaccaactgtcttccgtctctcaggctaggaggag

SEQ ID NO: 66 - DNA, 87 bp, Artificial Sequence
  Synthetic Construct
ttctagcgatcttctgtcgtctcaactttcgtcatgggacctgcagaggtcatctcatgtcgcatgtcgcatccattccgtcgaatg

SEQ ID NO: 67 - DNA, 87 bp, Artificial Sequence
  Synthetic Construct
ttctagatcaagaagcgcaatgcagacctctgcaatttgttacgcaattcgtacgattactcgagacgctgaacgacacctaagtgc

SEQ ID NO: 68 - DNA, 87 bp, Artificial Sequence
  Synthetic Construct
ttctatcgtatatatcgtgtcatgacatgcttggtcgacgaggtcggaactagcatcgcaggcacgcacacggatccagatcgagct

SEQ ID NO: 69 - DNA, 87 bp, Artificial Sequence
  Synthetic Construct
ttctagacttcacatcaccacaatgacgcgagacagttagctccgaaggtatcgcgattgccagctactggactcaacgtatatgct

SEQ ID NO: 70 - DNA, 87 bp, Artificial Sequence
  Synthetic Construct
ttctagacaatacagtgttctacattctaccatcgttcggagcctcagaagctgaatatcgctactatcatactctcaactatcacg

SEQ ID NO: 71 - DNA, 87 bp, Artificial Sequence
  Synthetic Construct
ttctagaactagatgtcttgaatgcgcttcactttctagcgatagcagaagatcgcgacagcaactatcagactccagtgccgatct

SEQ ID NO: 72 - DNA, 87 bp, Artificial Sequence
  Synthetic Construct
ttctagaagtatccactgaatttccacaagttcagtcatacgagcggtgtctctttccgtgcagagtcgagagtaacatgaatccat

SEQ ID NO: 73 - DNA, 87 bp, Artificial Sequence
  Synthetic Construct
ttctagagtcgatgacattacggacgattgagcggaacaaatgaggcttgattaagacgatagcgacacgtcacttctagtgtgttc

SEQ ID NO: 74 - DNA, 87 bp, Artificial Sequence
  Synthetic Construct
ttcctcgtatgcgcacgagtgcagggactccctcagatcgtctatggtcatgatatagatgctctccctgagacgggagtggtatga

SEQ ID NO: 75 - DNA, 87 bp, Artificial Sequence
  Synthetic Construct
ttctctgcgatatgtttagaccgtctcatatagttctgattcccatctggtgtgctcaaggtgccttgtgctttatagaagtcaggt

SEQ ID NO: 76 - DNA, 87 bp, Artificial Sequence
  Synthetic Construct
ttctctgctgagttctcatatagtagcgacgtccatcgcttgtgaaaggcatatctattgaagcgcgtgacagctatctcgatgcga

SEQ ID NO: 77 - DNA, 87 bp, Artificial Sequence
  Synthetic Construct
ttctctagatactaggatacacagagttgattaacagcttatagatgcgacactacacgatagagccagctgtagctcaacgtcact

SEQ ID NO: 78 - DNA, 87 bp, Artificial Sequence
  Synthetic Construct
ttctctagttgcggttgactcgtgatgctagagggcgctagatcgaaggagcctatccgatctcgaactttggatccgatcttcctc

SEQ ID NO: 79 - DNA, 87 bp, Artificial Sequence
  Synthetic Construct
ttctctgtggtcgcgttcagccattctcagggaatggctggtctcgtgtactctaaggatcctactcctatgcctcgtagacagtga

SEQ ID NO: 80 - DNA, 87 bp, Artificial Sequence
  Synthetic Construct
ttctctgtctctaactcgctaaagctcagaaagcagtgtgtctcagtcgagaactctcgtatcccttgaccttgccgaaagctcgag

SEQ ID NO: 81 - DNA, 87 bp, Artificial Sequence
  Synthetic Construct
ttctctacgggtacatagaactgagtatacctgacgggtttgaacatcaatcgctatggactcccgtctgctcagatggtactagcg

SEQ ID NO: 82 - DNA, 87 bp, Artificial Sequence
  Synthetic Construct
ttctctacttctggattaagagctcgtgcggtatagggattctcttgaagtcctggcggcacttacatgagtgtaaacgcacagtga

SEQ ID NO: 83 - DNA, 87 bp, Artificial Sequence
  Synthetic Construct
ttctctaagttctctgtctctccgcatgcactcccgcatcgcctcataacagagcgattacgctgatgagctccgtagtgtcgttga

SEQ ID NO: 84 - DNA, 87 bp, Artificial Sequence
  Synthetic Construct
ttctctaacagaatgcgacagtagtacagaccataggactgtgattgactgtgtttcagacctagttcagtggtctagtgcatctca

SEQ ID NO: 85 - DNA, 87 bp, Artificial Sequence
  Synthetic Construct
ttcccgtacacaaacgtgactgcttactcttatactatgtctctcgtagagagaccaccagtcgtctacactgtcgtatgcgaggca

SEQ ID NO: 86 - DNA, 87 bp, Artificial Sequence
  Synthetic Construct
ttcccatcattccagttccacgagcctccgcgatgatagtcagacctatacagattctctcaggcattgaactgcgagtcgagtagc

SEQ ID NO: 87 - DNA, 87 bp, Artificial Sequence
  Synthetic Construct
ttcccgtgtaagcagatgataatctagtcagcaatcggtagctagaacatcgtcagcactataagtcatagaactcgaacttctaag

SEQ ID NO: 88 - DNA, 87 bp, Artificial Sequence
  Synthetic Construct
ttcccatagagtcgaatgtcatagttccacttaagaagatgtactatccgagaggcggagataactatcaagatgacactcatggtc

SEQ ID NO: 89 - DNA, 87 bp, Artificial Sequence
  Synthetic Construct
ttcccattccgcttccatcgcgcacacgagagatgttgctctgagttagtggtccattgtggaggactccgacgctagcgtagaaag

SEQ ID NO: 90 - DNA, 87 bp, Artificial Sequence
  Synthetic Construct
ttcttgaagccgcctttccagaatcctgtacaggtgcatgctaagtgcgtaacttagagtaactacctaggtacgatctgacgacag

SEQ ID NO: 91 - DNA, 87 bp, Artificial Sequence
  Synthetic Construct
ttcccatctacgttcggtaagtgtactccgccttcgtctgacgagcgatagagatatacactaccgtacctggtccactaggcactg

SEQ ID NO: 92 - DNA, 87 bp, Artificial Sequence
  Synthetic Construct
ttcccgttagtgtatacgcgaatcatccagactaaggcaccatagccactcgtcccggcatatctagtaaatgtccgcttaataaag

SEQ ID NO: 93 - DNA, 87 bp, Artificial Sequence
  Synthetic Construct
ttcccgctctctctgcagatctacgagctcccgcgacgaagtgatttcactcgccgaggattacgcccatgtttcctaggatcagcg

SEQ ID NO: 94 - DNA, 87 bp, Artificial Sequence
  Synthetic Construct
ttcccgtgaagagatcgaggacatcatactagcaagttgtgtgcattgttcgtgggaatccgaccttattcgtagtagtcgctgtga

SEQ ID NO: 95 - DNA, 87 bp, Artificial Sequence
  Synthetic Construct
ttcccacgtcgcagccgaagtaagtaggtgagactactaggacgccgtgatccagatttggctacttgatagaattgaagaaaggtg

SEQ ID NO: 96 - DNA, 87 bp, Artificial Sequence
  Synthetic Construct
ttctcgagaagaagccatgcgtgtctgaagtgaataatgggcgtcgtccctccggacacgagcacgccatcggctgagcagagtccg

SEQ ID NO: 97 - DNA, 87 bp, Artificial Sequence
  Synthetic Construct
ttctgttctgactagagttaggctatgttacagatgccaggtaagactcgtctcccgttatattaggagtctacttagtcatataga

SEQ ID NO: 98 - DNA, 87 bp, Artificial Sequence
  Synthetic Construct
ttctgttcaccttcaggacagctgccggagctcagactacgaagagaccctggcccgttctcacgtaagcgatgcagtagtaacata

SEQ ID NO: 99 - DNA, 87 bp, Artificial Sequence
  Synthetic Construct
ttctgcttcttgaatacacagtctacaaatgtctatgtgacgggtagaggcgctactcgctcattacgccagccacgaatcggaagt

SEQ ID NO: 100 - DNA, 87 bp, Artificial Sequence
  Synthetic Construct
ttctgtttgttgtcaggctgatagcgatgcggccctctctgcaacacggagacaagatcgtctgagctccacggtccgcctcctgca

SEQ ID NO: 101 - DNA, 87 bp, Artificial Sequence
  Synthetic Construct
ttctagggtctcagcacggtggcgttcgcataggtgagttacaagggccgtctcagatcgatcgtaatctcgtgctgcgtaagcggt

SEQ ID NO: 102 - DNA, 87 bp, Artificial Sequence
  Synthetic Construct
ttctagggatagcatatctagccattctagtagtctttcagtagactgatcgacgcaagcgtggagagaaatcgccgcggctgagct

SEQ ID NO: 103 - DNA, 87 bp, Artificial Sequence
  Synthetic Construct
ttctaggatatgggattcttgcgactcagaaatcacgatgcgcgtgaggatgagcagaactctccgcagctcggctattctccggtg

SEQ ID NO: 104 - DNA, 87 bp, Artificial Sequence
  Synthetic Construct
ttctaggagcatggactcatagagcctcgagtaatgctagtcggttgccacttaggaccaacacctcagtagcagccttgaccagtc

SEQ ID NO: 105 - DNA, 87 bp, Artificial Sequence
  Synthetic Construct
ttctaggctaacgctatctgtggaacatctaagagatcggatatattcagacagccgagcctaagcatcatcgatggattcctcgct

SEQ ID NO: 106 - DNA, 87 bp, Artificial Sequence
  Synthetic Construct
ttctaggcagtggtaagtgtagagtcatatcctgtgcacagagtcccgtgtctcgtattgcagggttcaatccagaacctattagtc

SEQ ID NO: 107 - DNA, 87 bp, Artificial Sequence
  Synthetic Construct
ttcttgagtctagagactctcctgggtaagtgctagtgtcataactattgcctgactcagctcactgtctcgcactagaacatcaga

SEQ ID NO: 108 - DNA, 87 bp, Artificial Sequence
  Synthetic Construct
ttctcaacactgagtgtattctctggagaggaccgtatatcgatcgtaacggagcctaagacgcacaatcctctgcgctctaagtag

SEQ ID NO: 109 - DNA, 87 bp, Artificial Sequence
  Synthetic Construct
ttcccgcgatcggcaacacgaccggagagaccaactcaggataatacgtgccagcctcgcctgcgtttccgtcgccgttgcgtacag

SEQ ID NO: 110 - DNA, 87 bp, Artificial Sequence
  Synthetic Construct
ttctcaaatggtacactggagaagccagacaactcttctcatcctggatcattacgtcctgatactagtgcggtcctcacgatgcag

SEQ ID NO: 111 - DNA, 87 bp, Artificial Sequence
  Synthetic Construct
ttctcaataagatgacatctgttgtagctcctcgtgacttagttgagccgacagccagagctcactgcacgagagagcgaggagcta

SEQ ID NO: 112 - DNA, 87 bp, Artificial Sequence
  Synthetic Construct
ttctcaactttgatcacatctggagtctagcagctgggactatagcctaagtcttcgctgctcggatgaaagggtcataaccgtatc

SEQ ID NO: 113 - DNA, 87 bp, Artificial Sequence
  Synthetic Construct
ttccacccttcttctccaccgatcttatgcgtaatcgtccgaggccatgatcaggtctgactcctcagaggtgagcgagcaggccct

SEQ ID NO: 114 - DNA, 87 bp, Artificial Sequence
  Synthetic Construct
ttcccaataatatgaagaaagccgagttatagacctttcttcgctgagaaggctaagcagtgagtcggcaacggtctaaatcacaag

SEQ ID NO: 115 - DNA, 87 bp, Artificial Sequence
  Synthetic Construct
ttcccgactatcagacgcaagctgcagcagcactagactttcaagctacgagacatgacgatcctccactgacgcttaagagatcac

SEQ ID NO: 116 - DNA, 87 bp, Artificial Sequence
  Synthetic Construct
ttctgcgactcttagtctatgttaatcggttattcaccttcaaatgtgcctccgagtcgcttattggctgacagcagtggcttaata

SEQ ID NO: 117 - DNA, 87 bp, Artificial Sequence
  Synthetic Construct
ttcctcgagacacctaagccggcttattgagctgatactatcgaggtgggatcagatctgcctcgttacgcagagtagggcatcgga

SEQ ID NO: 118 - DNA, 87 bp, Artificial Sequence
  Synthetic Construct
ttcctcagaatcggacatcgcctgcatctcatggagctatgaatattctctgtcggccagcacctaaagagacaggatggccgcgag

SEQ ID NO: 119 - DNA, 87 bp, Artificial Sequence
  Synthetic Construct
ttctcaccttctcagctaggtgtcacgactctgcagtagcaggcgtatgtacgctgtccgccgcatggcttgactctcgtagagctc

SEQ ID NO: 120 - DNA, 87 bp, Artificial Sequence
  Synthetic Construct
ttctcactggtcactggacagagtccacgcactacttatcagtagggaatctgcgtgtctactttgatgccgtagcagctgtaggga

SEQ ID NO: 121 - DNA, 87 bp, Artificial Sequence
  Synthetic Construct
ttcttcgagctcccaatctatgactgactcatcagagctacgccgtgtccaaacccgaagtcaccagcgccatcacgacactatctc

SEQ ID NO: 122 - DNA, 87 bp, Artificial Sequence
  Synthetic Construct
ttcttcgacctagtgggattgtgactgcagctgcgattcataggaaatgctttccacgatgtctgattctacggtttcgtcctcgga

SEQ ID NO: 123 - DNA, 87 bp, Artificial Sequence
  Synthetic Construct
ttctcgcgtactcctcagtcttaggtatagaagtattgctgattactgcgtctgcactagtagttcgatccgttccgtttccagctc

SEQ ID NO: 124 - DNA, 87 bp, Artificial Sequence
  Synthetic Construct
ttctgaagacctctcgctaatctctatcgtctaactctatcttagggacgcctctagctagcagtctcgctaaaggctcgcgaggat

SEQ ID NO: 125 - DNA, 87 bp, Artificial Sequence
  Synthetic Construct
ttctcgcatagcccgcgaatgcgtgtgacttagtgcatccagagtcctatgccttcggtcaatggacacatagtcgtctgagatact

SEQ ID NO: 126 - DNA, 87 bp, Artificial Sequence
  Synthetic Construct
ttctcaccggagcgacgtatattagctcacctacctcactatcagtgaggaatgcagcctgtgggcgcttgacagcattcgaagaag

SEQ ID NO: 127 - DNA, 87 bp, Artificial Sequence
  Synthetic Construct
ttcttcagactgcacacttctacaccagtctgcctaaagcagatcacacagtagagatagctctctgtcactagtctatattatgag

SEQ ID NO: 128 - DNA, 87 bp, Artificial Sequence
  Synthetic Construct
ttcttcagcactgctgtgtctggctctagtggtaatcgaaaccagatggtcaagatctaggaggagcgcagatcaaatagatcgaga

SEQ ID NO: 129 - DNA, 87 bp, Artificial Sequence
  Synthetic Construct
ttcttcaagcgaagcagacgaacgtagactactctgtgtcaggcatgccgctgacgacagactcagccgcagccttgtggtctatag

SEQ ID NO: 130 - DNA, 87 bp, Artificial Sequence
  Synthetic Construct
ttctcacgagtagagagtcctcgaaagctcaacaatcgtgacagaaacggatagtcgcacataacattcacaacacctgcaatgctc

SEQ ID NO: 131 - DNA, 87 bp, Artificial Sequence
  Synthetic Construct
ttcttcgcaggaatcacatcacacccgtacatcgcttagcgacaggtgttatgatgaaatttctacggccacctggagtctggagca

SEQ ID NO: 132 - DNA, 87 bp, Artificial Sequence
  Synthetic Construct
ttcttcgctctcatatactgacgaactcgcagctcgcacagccaccgaggcacgcgctgatctgagcacgctgtcgcagcattggag

SEQ ID NO: 133 - DNA, 87 bp, Artificial Sequence
  Synthetic Construct
ttcttcgtactatgacgactccatgcgtagaatttctgagctaatgatctacgagacttgccattcagagcgatccgacatagaggc

SEQ ID NO: 134 - DNA, 87 bp, Artificial Sequence
  Synthetic Construct
ttcttcgtccatctcgtatgtcgaaagtattgtagcagtctcccttgcagcgcgttatagtcattgcatgtcactatgttcgtaaga

SEQ ID NO: 135 - DNA, 87 bp, Artificial Sequence
  Synthetic Construct
ttcccaatcgtcagagcttaggtagacactttcgtcacaacatgacatatgaaggtagagtatgagtgcccatcggtcataatctgt

SEQ ID NO: 136 - DNA, 87 bp, Artificial Sequence
  Synthetic Construct
ttctatatcgagtacttcggccctgcggacactgcttacaagcgaataggccctggtgcggtcgtcctcgtcctaggaagagactcg

SEQ ID NO: 137 - DNA, 87 bp, Artificial Sequence
  Synthetic Construct
ttcccacctaagcagtagtgacgattagtaccaacacattgacgagacaagtgaggtctatacaatataaatgtacgactctcaaag

SEQ ID NO: 138 - DNA, 87 bp, Artificial Sequence
  Synthetic Construct
ttcccagagcctctaacagtctgctagtgcagctgaacttgactgatgtgagatggttcaataggtggcttaatagcacgacatgga

SEQ ID NO: 139 - DNA, 87 bp, Artificial Sequence
  Synthetic Construct
ttcccacacagccagttacctctcgcagcgggacctgtgaatggcttaagaatgcacgtaatccgttcttgattccctgagacttca

SEQ ID NO: 140 - DNA, 87 bp, Artificial Sequence
  Synthetic Construct
ttcctcggaaacctacctaagtgccatccttagccatgactcaacggaatcaatgtcggctatactcctgcaactgcttgctacccg

SEQ ID NO: 141 - DNA, 87 bp, Artificial Sequence
  Synthetic Construct
ttctcagataagtgacacgatcagttcgcattcaattgtaagcctttaacagcttagtaggtcttctagatctctgcgtacacgcca

SEQ ID NO: 142 - DNA, 87 bp, Artificial Sequence
  Synthetic Construct
ttctcggagcgcaacacaaatagtaagtctctccctgctgcacagcataagtataatttcaagaagttgcacacttcacctctcccg

SEQ ID NO: 143 - DNA, 87 bp, Artificial Sequence
  Synthetic Construct
ttctcgggtcacgcaaacgtgacatgctgccctagattctgcacggagcgtaacgcttcttacagcgctgtcagcagcacttcgcgt

SEQ ID NO: 144 - DNA, 87 bp, Artificial Sequence
  Synthetic Construct
ttctcgggacacggtggtactctaggcgataagtgcgtcacacgcgcatgtccttctgctcatttctagctcgctgacatgggtcct

SEQ ID NO: 145 - DNA, 87 bp, Artificial Sequence
  Synthetic Construct
ttcctcgacgtcagactatataagtgaagagcgccggcggtatagtctcacgcaaagactaagccgtcagtcagcgctggactcgga

SEQ ID NO: 146 - DNA, 87 bp, Artificial Sequence
  Synthetic Construct
ttcctcgcggagctatctgagacaaatccttagccgcagtagagccagcagatccgcatcatcgtgttcgcgtctctctactagaag

SEQ ID NO: 147 - DNA, 87 bp, Artificial Sequence
  Synthetic Construct
ttctattctagttagtacgatgagcagtactgaagagagctggtgagcctcaagtgtatgtatataggcgagcacctaagtataaga

SEQ ID NO: 148 - DNA, 87 bp, Artificial Sequence
  Synthetic Construct
ttctactcgggaatactgcgaaacctatctcgaggactagcagtcgagagagtagagcctgatttcttcgctggttacgatagtgga

SEQ ID NO: 149 - DNA, 87 bp, Artificial Sequence
  Synthetic Construct
ttctactatcgacattatgatgtggatcacttaccagtacatcctggaactaacttatgaaagcagtagtcttacccacctggtggt

SEQ ID NO: 150 - DNA, 87 bp, Artificial Sequence
  Synthetic Construct
ttctgcgcggtgtgtgtaagatacgcttaggctgtcccactccactgtttgggtacgtcaactggtaagtcgaagaagtgaagagca

SEQ ID NO: 151 - DNA, 87 bp, Artificial Sequence
  Synthetic Construct
ttctgtgctgagtaggcggaggcttcggaccctttctctgtcggagcgcagttattacgacgctctcgacgaaagtctacggataag

SEQ ID NO: 152 - DNA, 87 bp, Artificial Sequence
  Synthetic Construct
ttctgtgtagacggcgtccagttacctgcaggctcatctacgacagattagttggctgcgctccctgtctgtctcagcggtggcccg

SEQ ID NO: 153 - DNA, 87 bp, Artificial Sequence
  Synthetic Construct
ttctgattcggtcgcgcgtataatttcaattaccgaggaatgagagtagtagactgacgcgacgatcctcgagacatgggatcgtct

SEQ ID NO: 154 - DNA, 87 bp, Artificial Sequence
  Synthetic Construct
ttctgtggagtctgatgtctgtctgagtgtgattcggcaatccagcacccagagctggcggcttgtccttatgataatgtggaccag

SEQ ID NO: 155 - DNA, 87 bp, Artificial Sequence
  Synthetic Construct
ttctgcggctctgtatatgtccagcgattccagttcgtgttctactagaatgtgttacgctgatatcgagctcatcacgagagattc

SEQ ID NO: 156 - DNA, 87 bp, Artificial Sequence
  Synthetic Construct
ttctgcgagccgaagaattgccgaccaataaagtctccgatcactcctgactctactgtcttgtcgcgccgagctgagttactgtcg

SEQ ID NO: 157 - DNA, 87 bp, Artificial Sequence
  Synthetic Construct
ttccatacttctatgccttcgtgagagtgcactgcaaagctacgtttccctttgctgtctcagacaagcgcgcaggctccgcactat

SEQ ID NO: 158 - DNA, 87 bp, Artificial Sequence
  Synthetic Construct
ttcttcatactgctcggagtctcgtatatcataactaagcatgattattacatcagacacagaaatgagtagttagcatctgcagct

SEQ ID NO: 159 - DNA, 87 bp, Artificial Sequence
  Synthetic Construct
ttcccagcgaaccacacaatacgaaactgcggtctcggaccgcagttcttcgacgatagaaagagtggaggaggagtaggatgacga

SEQ ID NO: 160 - DNA, 87 bp, Artificial Sequence
  Synthetic Construct
ttcccaacggtatagtgagctctagtcagcaagctggagatccgtttaagcttctctgactgaacagcgctgctgacagcagtgttc

SEQ ID NO: 161 - DNA, 87 bp, Artificial Sequence
  Synthetic Construct
ttcttctgctgaggactcgtgactcagcagctgtgctatacgagacgaaagaatactagaggactcctccatgcagcttgaacgctg

SEQ ID NO: 162 - DNA, 87 bp, Artificial Sequence
  Synthetic Construct
ttctgttacatggacgctgcacagtgtcgtaagagacgatgtccgttatcgctcggttagctcttcgctggccctatctcgtatagc

SEQ ID NO: 163 - DNA, 87 bp, Artificial Sequence
  Synthetic Construct
ttctgttaggaggagcctgctctaactccgagaagactacagcgccgagcacagacaagatgagatcatccggctacacgcgtccgt

SEQ ID NO: 164 - DNA, 87 bp, Artificial Sequence
  Synthetic Construct
ttctgttgcggtgcgctcatcacttacccatgcgtggtgggatctcgtgctaacatgttgtgtatcctccagaagtcgccttatgtc

SEQ ID NO: 165 - DNA, 87 bp, Artificial Sequence
  Synthetic Construct
ttctgctgacattgcgtccctccttcaggaggatctataagccactctcgaataccgctaatacaccgccgaatcgctctaagtatc

SEQ ID NO: 166 - DNA, 87 bp, Artificial Sequence
  Synthetic Construct
ttctgcctctgtcacactgaggagcctgctcctccttgcggacctactacttctagagagcgactctgtataggcttactaccggct

SEQ ID NO: 167 - DNA, 87 bp, Artificial Sequence
  Synthetic Construct
ttcctccctctcgacttatagacgatggaggctacttgctcgcacggacagcagtatcgtgatctgatggtcctaatgaatttagag

SEQ ID NO: 168 - DNA, 87 bp, Artificial Sequence
  Synthetic Construct
ttctgtcctgagcacactgcttgtccacgcagtgtacgaaaccacctgagatctacttgaggcacgctcaacaacgcatgagtcgca

SEQ ID NO: 169 - DNA, 87 bp, Artificial Sequence
  Synthetic Construct
ttctgcccgacgagttgttgctaggtctgattccacggtgtccctgagtgactggtcgtacgcctcctagcgctcttatcttgcaat

SEQ ID NO: 170 - DNA, 87 bp, Artificial Sequence
  Synthetic Construct
ttcttcatcagaactataggaactacatgtgtggacaagtgctagggaggcggcatgcctcgttcgacttatggttagaacgcgcag

SEQ ID NO: 171 - DNA, 87 bp, Artificial Sequence
  Synthetic Construct
ttctgccagatcgagagcggactgcataacctatctaaggcgtctgtcaaggagactatgctaggactcgagggacacttcaagaag

SEQ ID NO: 172 - DNA, 87 bp, Artificial Sequence
  Synthetic Construct
ttctgaccaggcctcttatcgtagatgcgtggaaatgacttacctctctagcagatgtctaatctgagatgaacttaggtcacatta

SEQ ID NO: 173 - DNA, 87 bp, Artificial Sequence
  Synthetic Construct
ttcttggaggcttgctctcactctaagctcttccctggcgcatactgatatatgaacgcatgagctgtcttctataagccggattgc

SEQ ID NO: 174 - DNA, 87 bp, Artificial Sequence
  Synthetic Construct
ttcctcctcttctatctctcatcatacagcagaagctgtctacgatcaaagctgagtactttcagaggcaagctggcgttctatgtc

SEQ ID NO: 175 - DNA, 87 bp, Artificial Sequence
  Synthetic Construct
ttcctcctgctcccgagatatcctatccagacgcctagttcgtatactaacggtcctgtacgaagcgcatagatagaggctaagatg

SEQ ID NO: 176 - DNA, 87 bp, Artificial Sequence
  Synthetic Construct
ttctcggcaacttagttgggctatttccgcgctcgagtaagaatgttaggagcgggatagctcggatagactatctgcggctcactc

SEQ ID NO: 177 - DNA, 87 bp, Artificial Sequence
  Synthetic Construct
ttcttccgacgacgaatctagggattccagagcgtcgcactatgccatccacctagcgagagaactggcgcagtggatccggcgaag

SEQ ID NO: 178 - DNA, 87 bp, Artificial Sequence
  Synthetic Construct
ttcctctgtactgctcctatcgtcatcgtccctctcctgttgatctatggttagcagatcactggaataccgaatccttatgtctag

SEQ ID NO: 179 - DNA, 87 bp, Artificial Sequence
  Synthetic Construct
ttcttactctctcgatcaaatgtcgcgctgcgtttgaactgatcaatgttacgtgaggcagtacgctctttccataaccgcttcata

SEQ ID NO: 180 - DNA, 87 bp, Artificial Sequence
  Synthetic Construct
ttcttatgagtcggccctggatctctcaagcagtagtgtgattagatgtcaaatggactctctatcctagagtctggaagaatcatc

SEQ ID NO: 181 - DNA, 87 bp, Artificial Sequence
  Synthetic Construct
ttcctctgatatggaccttatagctgtcactcatgctatttagcgagagctgtactcttcaagtcacgtctaccttgaagtctgtat

SEQ ID NO: 182 - DNA, 87 bp, Artificial Sequence
  Synthetic Construct
ttccctacgaatttcccataggatttacagaaggcaaagactagaactcgatcgagacagcgatctcgaatgttcggaaacctcaag

SEQ ID NO: 183 - DNA, 87 bp, Artificial Sequence
  Synthetic Construct
ttccctactgaggctcgcggcaacccggctggctagacaaatagcgcgcagctaatcatgactcagttatcagatctcgattgttat

SEQ ID NO: 184 - DNA, 87 bp, Artificial Sequence
  Synthetic Construct
ttccctatgccagagaagtgagagcgcgtgatactaggagagttgggaagaactataccggctgcttagtgtaagagaagttgacga

SEQ ID NO: 185 - DNA, 87 bp, Artificial Sequence
  Synthetic Construct
ttccctatctgaactaagcctcgactccgagctactaatggctactacaacagacacaagagaagaaagtctatcctacgtctggct

SEQ ID NO: 186 - DNA, 87 bp, Artificial Sequence
  Synthetic Construct
ttccctcgacacagctgtctcttagatacgactgcaggagagacagactagttgtgaatcggagagtgactagtcgtgacgatcgat

SEQ ID NO: 187 - DNA, 87 bp, Artificial Sequence
  Synthetic Construct
ttccctcgtagagctaagtctatcgctgacaataagtgtacttacgagaatttaggccattcaggtacacgactagtcatgcgtagc

SEQ ID NO: 188 - DNA, 87 bp, Artificial Sequence
  Synthetic Construct
ttccctcagtagggtagctgttctcgatatactcacatgaagactcctctctaggagccacctcgagcattcatgaacgagactggc

SEQ ID NO: 189 - DNA, 87 bp, Artificial Sequence
  Synthetic Construct
ttccctcatatattaccagtgcgactccagttcactgtccgaagcgcaatcgctttggtagacggtcacgtcgtccatagacctgtc

SEQ ID NO: 190 - DNA, 87 bp, Artificial Sequence
  Synthetic Construct
ttccctccgtatgtgttagcaagcctaaagaatttgaagagattgtgccgtgcgtatgatcacggattcgcgtgcgagtgtgtgtag

SEQ ID NO: 191 - DNA, 87 bp, Artificial Sequence
  Synthetic Construct
ttccctcctcagggatgaatctacttcgtgcattatccttctcagaaccaccactactcgtagacaatcagacacggttagtacgca

SEQ ID NO: 192 - DNA, 87 bp, Artificial Sequence
  Synthetic Construct
ttctgagactgacagcagagactcgatggccagtgaaagttgagaactcgttgagctcagtaggacttcaactctcgatctccgcct

SEQ ID NO: 193 - DNA, 87 bp, Artificial Sequence
  Synthetic Construct
ttcctctcttattgcgcgatcgctgagcctcgttagatgtgcgaccatatatcttgagtggtagtgtctggaccagaggcgaaggtg

SEQ ID NO: 194 - DNA, 87 bp, Artificial Sequence
  Synthetic Construct
ttcctctcgagaggatgacattctggtcataatccgaagttccgttctactcctctcgacatagtcctgactatcacgccgaagatc

SEQ ID NO: 195 - DNA, 87 bp, Artificial Sequence
  Synthetic Construct
ttctgtctgttgtgcataagacgatatctcgtcatgcatagagtacagcagttcttccgaatctaggagtacatggtcaacacaagc

SEQ ID NO: 196 - DNA, 87 bp, Artificial Sequence
  Synthetic Construct
ttccattctaatctgaagtatactagctgcttgagaaatggatctcaggcaatgaagctaccatgcgtgttaatcctacgagacctc

SEQ ID NO: 197 - DNA, 87 bp, Artificial Sequence
  Synthetic Construct
ttccactcggtgcatgcatgagctagttgccgacgcagacgccctagcagtacagcgcgaccaacactcggattcaactgagctaag

SEQ ID NO: 198 - DNA, 87 bp, Artificial Sequence
  Synthetic Construct
ttccattacaatgcactgggaggattgtgtgcacagcatgagatactacctaaggctcctctccgatagtcttcgtctccagagccg

SEQ ID NO: 199 - DNA, 87 bp, Artificial Sequence
  Synthetic Construct
ttccattagctgaacgtgcagccgacatgctacatcccgtcgacaagccctccaacttgtgaggagcagtagccttagttcctcttc

SEQ ID NO: 200 - DNA, 87 bp, Artificial Sequence
  Synthetic Construct
ttcccgggcctcgagttcggttctaactgccaggctatcaacttcgtcgacagccgactgaaggagttcagttagggaactgtgcta

SEQ ID NO: 201 - DNA, 87 bp, Artificial Sequence
  Synthetic Construct
ttctcggtccgaagatcttagtgctatgctcctggagatggcagatgtgcgacaggattgtcacatgctagtggactccgtcgtagt

SEQ ID NO: 202 - DNA, 87 bp, Artificial Sequence
  Synthetic Construct
ttccacttcctgatctctccgcatgcttgtcctggtaagacaggaacaagccgctagggttagggaagcgagtgtgcttgtggagct

SEQ ID NO: 203 - DNA, 87 bp, Artificial Sequence
  Synthetic Construct
ttccatttgtgagcgtgaaagggcatctgtgaggcatctttcgagtcattcagaagcgtccatactaagtctgaggtccatggtcga

SEQ ID NO: 204 - DNA, 87 bp, Artificial Sequence
  Synthetic Construct
ttccactgtggactattcggatcagcttgcctctcattattgatcagcttcagctgaacgtaggtctacttggtctcgtagttagct

SEQ ID NO: 205 - DNA, 87 bp, Artificial Sequence
  Synthetic Construct
ttccactgaagatctgtccacaagggttgttgaaacccactgtgaccggcgtgattgagagatcgtcagggtaatttgccgcgacga

SEQ ID NO: 206 - DNA, 87 bp, Artificial Sequence
  Synthetic Construct
ttctctcatagatcatatcgtcgaatcgctactctactggctctcatattatatagagtgtcttgaatgctgactcgcactttgagc

SEQ ID NO: 207 - DNA, 87 bp, Artificial Sequence
  Synthetic Construct
ttctgtcacaaggtcacgttcgatcgcctgataggaccaccgtatgagactcacggtacgcagctctctgtcgtagctcatgtggag

SEQ ID NO: 208 - DNA, 87 bp, Artificial Sequence
  Synthetic Construct
ttctctcgttagtctgctttcgagcagcgtagagataattgaggcttctctgagaagtcttgactccgatcactattctgctatgag

SEQ ID NO: 209 - DNA, 87 bp, Artificial Sequence
  Synthetic Construct
ttctctcgagcacgttacctcgtcctcgcatcacaggtatcataggtacgatgacctgagcaccaggtcgatagtaatgtgccagac

SEQ ID NO: 210 - DNA, 87 bp, Artificial Sequence
  Synthetic Construct
ttctctctcgtcccgtcggtccgaatgtagccgacacgaatcatcgcgttggctcgaactggtcgatgaagttgagcgcgaagaatc

SEQ ID NO: 211 - DNA, 87 bp, Artificial Sequence
  Synthetic Construct
ttctctctgcctggctgaggctaccctcctcagatattcccaatgtgagatgtctcatataagatatatcatcacaagcgaccattc

SEQ ID NO: 212 - DNA, 87 bp, Artificial Sequence
  Synthetic Construct
ttctctcctggaggattagtagtctatttgacgaacctagctgacctattaggaggttctctcgcaagccatggcacactgtcgtgc

SEQ ID NO: 213 - DNA, 87 bp, Artificial Sequence
  Synthetic Construct
ttctctccgctctcacagcgctcaggaactccatgatgatcttgccgaccagtagtatgaaatctcaactaccgatacgcagtaaga

SEQ ID NO: 214 - DNA, 87 bp, Artificial Sequence
  Synthetic Construct
ttctctatctagccaatcacggcacactgaagcgctcagcagacgccgtacgtgtacactgtgccttgtctcatatgcactacatct

SEQ ID NO: 215 - DNA, 87 bp, Artificial Sequence
  Synthetic Construct
ttctctatacacggactccgactgatccctgctaaggagggtttctagcctatctcgagactgccttagcacacaactgaggtaatc

SEQ ID NO: 216 - DNA, 87 bp, Artificial Sequence
  Synthetic Construct
ttcctccgatacaagttgataatcctcctggagcctttcaaggagagtcctatcatccagttggatttagagaagggtcgattaaag

SEQ ID NO: 217 - DNA, 87 bp, Artificial Sequence
  Synthetic Construct
ttcctccgtttcgctatccacttgttcctccctcgacataagataccggtcagagcttgacgcggcagaccgttccgaaacctcgtc

SEQ ID NO: 218 - DNA, 87 bp, Artificial Sequence
  Synthetic Construct
ttcctccagggaatggctaagcgcgtaactcgcctctgagctccgctggtattacctcgaagacgtgtcgtcctctatactcgagct

SEQ ID NO: 219 - DNA, 87 bp, Artificial Sequence
  Synthetic Construct
ttcctccacgtgttcgcaggattattactaatccgaagaatccgttcacagctattcgctcgaactggacgccataattaggtcctc

SEQ ID NO: 220 - DNA, 87 bp, Artificial Sequence
  Synthetic Construct
ttcctcacgggcatccgaggatgctcttgatgagagatgggaatgctggaggattcagactgttcacaggtgtgctgacctatgaga

SEQ ID NO: 221 - DNA, 87 bp, Artificial Sequence
  Synthetic Construct
ttcctcactgtgcgtgaccctaacgcgggaaataacactagattgaagggattattaaacatcagagtgtagaaggcaagcactgct

SEQ ID NO: 222 - DNA, 87 bp, Artificial Sequence
  Synthetic Construct
ttcctcatgatcaagtgatcaaatcagcgatatagagtcttctgcagacagttcggccatgaggctgcgtataagttacatccacca

SEQ ID NO: 223 - DNA, 87 bp, Artificial Sequence
  Synthetic Construct
ttcctcatctatacacctaacgcgtataatacgcgagagggccctggatgtctacaggtacctgtcatccgagaggtaaaccatagc

SEQ ID NO: 224 - DNA, 87 bp, Artificial Sequence
  Synthetic Construct
ttcctcaaggcttgtcgaagtgcgatattcgaggcgctcgtcgctcgatatttctgccgataggcgagagtaactctgtcacctcgt

SEQ ID NO: 225 - DNA, 87 bp, Artificial Sequence
  Synthetic Construct
ttcctcaacttcgtaaagagagatccgtcattctctactgagttacgagacacattcctctgaagagcggaccgtgaccagactcct

SEQ ID NO: 226 - DNA, 87 bp, Artificial Sequence
  Synthetic Construct
ttcttgcgtctataggtgtctagtatcatcacactacctacttgagctcgtgtccctgtccaggtgctcctcgtgtgattagtctct

SEQ ID NO: 227 - DNA, 87 bp, Artificial Sequence
  Synthetic Construct
ttcttgcaggcgataacagtctgaatatagtgctgcgatcagttaaagataacgcgctgaggcgtcaagacgggctctgatccatgt

SEQ ID NO: 228 - DNA, 87 bp, Artificial Sequence
  Synthetic Construct
ttcttgatcttcgagtgaaactcacctaatgctagctctgctgtcgctcgtacgggatcattataccctttgacgacttaccaccag

SEQ ID NO: 229 - DNA, 87 bp, Artificial Sequence
  Synthetic Construct
ttcttacgaaatacttcaactgatgtatacacgtcgtctcgcagctgacgctgaggtctcgagatcaatcgtctccaggctcgtgtc

SEQ ID NO: 230 - DNA, 87 bp, Artificial Sequence
  Synthetic Construct
ttcttacctaagggactacgtgacgctacaaattacttcgatcgtcagcgaatcatctctcctaacggtgacagatcgactgtattc

SEQ ID NO: 231 - DNA, 87 bp, Artificial Sequence
  Synthetic Construct
ttcttactggatttgacgtactgagctgctgtagatcacatgcagttcgctttattctacgtattgactggtgtcatcgaggacgat

SEQ ID NO: 232 - DNA, 87 bp, Artificial Sequence
  Synthetic Construct
ttcttacactcactctaggcatcgaacggcatcggtgtccgattgtgtctcttagctgctacacctatacgtccttcgactggtgat

SEQ ID NO: 233 - DNA, 87 bp, Artificial Sequence
  Synthetic Construct
ttcttgccattctgtggctgaaacgcgcagaatagtagccctcagttctcaggtagactcggagcacaggagtcgggatatgagctg

SEQ ID NO: 234 - DNA, 87 bp, Artificial Sequence
  Synthetic Construct
ttcttgactctccattgattctctttcaagtatcgcttcggacaggcatgtatacagcaccgcgtcgcagcgacgatctgacataca

SEQ ID NO: 235 - DNA, 87 bp, Artificial Sequence
  Synthetic Construct
ttcttgatgtcacagacaggttagatgcgacgaaagtattatgcacgagtctgacgagtaagaagcctcactcctggacgaggattg

SEQ ID NO: 236 - DNA, 87 bp, Artificial Sequence
  Synthetic Construct
ttcttctacgtcgcgccttctctcgcaactggatgatgacatctcgagtcagcgtacagatagcgcaacgcgttctcaacgcgctga

SEQ ID NO: 237 - DNA, 87 bp, Artificial Sequence
  Synthetic Construct
ttcccaagcttcttgtcttcatattagtgctgactcctacctccacatcagcgccgaatcataactacgaacaagatcactatagtc

SEQ ID NO: 238 - DNA, 87 bp, Artificial Sequence
  Synthetic Construct
ttcttggcgagagctgatacttagcatgctacgcacctccgctgccacatctctagctgacgcctgtgtagctatcacatgacgtat

SEQ ID NO: 239 - DNA, 87 bp, Artificial Sequence
  Synthetic Construct
ttctgtgtctcatatatcctagctacagatacgatgtctctgatgccacctggagtgttgtctcgtggtctatatggacacataaca

SEQ ID NO: 240 - DNA, 87 bp, Artificial Sequence
  Synthetic Construct
ttcccgagattcttatcttcatactagtgttgactcctacctccacatcagcgtcgaatcataactacgaataagttccgaagccgt

SEQ ID NO: 241 - DNA, 87 bp, Artificial Sequence
  Synthetic Construct
ttcccaaagggtttgtatggaatcagttgcatcgtccgaactttcatcatatcgtatgctccacctaataataactagtaccgttga

SEQ ID NO: 242 - DNA, 87 bp, Artificial Sequence
  Synthetic Construct
ttctacagaagaccagctacttgagagactgtctacatcgtctcatgaccttcagtgcgccagaagtaccatcgcgtcctcctcctc

SEQ ID NO: 243 - DNA, 87 bp, Artificial Sequence
  Synthetic Construct
ttctacagctcgcgcggacgaaatcattcggtcctgcgacgtagatgagtcccaacaaacgtagatatctagcgacgaatcggtaag

SEQ ID NO: 244 - DNA, 87 bp, Artificial Sequence
  Synthetic Construct
ttctacaagtgttcttgaacaccagtgatcagcgcagctcagtctctaggagcaagacgagtctgactcacatagctcacggtccga

SEQ ID NO: 245 - DNA, 87 bp, Artificial Sequence
  Synthetic Construct
ttctataaccctagtaagtgtacgatctgagtgccgtctctgtctacgatctctcgatatgagccttcgccggcttgatcgatagta

SEQ ID NO: 246 - DNA, 87 bp, Artificial Sequence
  Synthetic Construct
ttctatacggtggcaagacgcgtcggacatctgactgagccaggctcgtgaactcattgatgaatcagaaagttcctagtcatactc

SEQ ID NO: 247 - DNA, 87 bp, Artificial Sequence
  Synthetic Construct
ttctatactggcactaaccaggtaagacgtctaccaggatagccgacttgcttcccatactgacgagactgtcagagattagatagt

SEQ ID NO: 248 - DNA, 87 bp, Artificial Sequence
  Synthetic Construct
ttctatataagagcgctcgactgaactgagccgcctcctgcaaacaactagactgtatgactcctaggaccgggcctctcgtcggga

SEQ ID NO: 249 - DNA, 87 bp, Artificial Sequence
  Synthetic Construct
ttcctgaagtgatattgaaaggtcagtcgtttcttcatgataggcgactatggattgtcgactatagagacttgtcagcacaagcag

SEQ ID NO: 250 - DNA, 87 bp, Artificial Sequence
  Synthetic Construct
ttctacgtgagtgctttcccagacaattattgaggtactcgacagcagactctcacagctgtggatactgcgacagaccctggttct

SEQ ID NO: 251 - DNA, 87 bp, Artificial Sequence
  Synthetic Construct
ttctatgtcttgcagggagtcggatgatagacgggccactgtgagctgaatggcgctgagaacgtctgtgtccactactgcactcgc

SEQ ID NO: 252 - DNA, 87 bp, Artificial Sequence
  Synthetic Construct
ttctgatctagtcagagcgctcgaggcagcctgagccagagacgcttgtagacgggacctatgagcgtgtcgcgaaagagagtcacg

SEQ ID NO: 253 - DNA, 87 bp, Artificial Sequence
  Synthetic Construct
ttctctgataatttcttaatcgagcaccctagaaatcacaactcaagtccaagtttcctaccgggatgatgactccgttcaggcaat

SEQ ID NO: 254 - DNA, 87 bp, Artificial Sequence
  Synthetic Construct
ttctcgaagcgatagctcctcagacctgcacgccgcagagatccgggacgaatggcttattctactcatgacccatgaaagcgagct

SEQ ID NO: 255 - DNA, 87 bp, Artificial Sequence
  Synthetic Construct
ttctgaaagaagaattatgaggcttagggatagtcgaagaagataccttgatagggagtcggttaggctcctagaagcactcacgta

SEQ ID NO: 256 - DNA, 87 bp, Artificial Sequence
  Synthetic Construct
ttctgaagttctcagcacttgtgatgcgcaaacttgggagcgcgtgagggttcaatgataactgacaatgcaacaacatactcgtac

SEQ ID NO: 257 - DNA, 87 bp, Artificial Sequence
  Synthetic Construct
ttctgacgaccgtgatgcgtcaacacgatcagagtccgcgcgtagtcacctctaaatccggaccgcctctgcccaccgttgaagatc

SEQ ID NO: 258 - DNA, 87 bp, Artificial Sequence
  Synthetic Construct
ttctgaatcgcgcacatgaagttgctgcatttgtactgaatctcacaggtggcaaagacggacggcctctcgctggtgtctgagcct

SEQ ID NO: 259 - DNA, 87 bp, Artificial Sequence
  Synthetic Construct
ttctgacaggcgtatctcttccctctcccatctcgtacattgggacctccgctcctctaggcatagttgtcgatccatgtcgaggca

SEQ ID NO: 260 - DNA, 87 bp, Artificial Sequence
  Synthetic Construct
ttctgacgttgagagtcttgattacagcagccactgtatagatacctcggcttgtagtgcagacgtcgccgaatcggtgctcagaag

SEQ ID NO: 261 - DNA, 87 bp, Artificial Sequence
  Synthetic Construct
ttctgaacaaatgagaatggaggagtgaacgtcccaagagcttagcgactagcagtccgactagcaactgacttcttcgcatctcag

SEQ ID NO: 262 - DNA, 87 bp, Artificial Sequence
  Synthetic Construct
ttctgaaatttcctaatcaacaagactcagtattactagccgtgttcgcgcggatgtacttgaaatgctaactacgctcgatgttct

SEQ ID NO: 263 - DNA, 87 bp, Artificial Sequence
  Synthetic Construct
ttctgaataagaggcgcggctactttgaaccagagagtctacgtctctgtagcgtcattatactcattccagagaacatgatgccga

SEQ ID NO: 264 - DNA, 87 bp, Artificial Sequence
  Synthetic Construct
ttctgaacttgcctctcttagttcaacagatgagcaacggagctagtggtctcaaagctcggcctccagcgcgctcgatactagcgc

SEQ ID NO: 265 - DNA, 87 bp, Artificial Sequence
  Synthetic Construct
ttctacggctgcactggacaggatatcccagactgatctcctttgaactgtcaggtcaatagaacactcagtatcatacgagatggt

SEQ ID NO: 266 - DNA, 87 bp, Artificial Sequence
  Synthetic Construct
ttctctttgggcgtcaaccgaggcctcatcacttcgacgggtctcatgcagtgcacgacgagaggaacttcttcactgctctatatg

SEQ ID NO: 267 - DNA, 87 bp, Artificial Sequence
  Synthetic Construct
ttcttattcgagcaggcatcgaagcgacgcataatcgctagagagctctctcgcactacgggcgatgtcatgactcgaaagaacata

SEQ ID NO: 268 - DNA, 87 bp, Artificial Sequence
  Synthetic Construct
ttcttcggagctctcgctttacagcctgctctgactgtcggtcacatatagagaaaccgccgcggagtcgagctctctagtctccag

SEQ ID NO: 269 - DNA, 87 bp, Artificial Sequence
  Synthetic Construct
ttcttatctgcttatactcgcgtcgatagaaaccagactttacctttagtcaaggtcgtccatagacgacctaactgtgagtagttc

SEQ ID NO: 270 - DNA, 87 bp, Artificial Sequence
  Synthetic Construct
ttcctatgagagccatctatgatagctctagcatcttgagctgagagagcggagctaaagcgactgtcattgcctctcgtgggatga

SEQ ID NO: 271 - DNA, 87 bp, Artificial Sequence
  Synthetic Construct
ttcttgttatgtagagatctcttatagctcatgaaccgtgcaggacgaaatgtggcaagacagcgcagaaagtgtcgcctgcgatct

SEQ ID NO: 272 - DNA, 87 bp, Artificial Sequence
  Synthetic Construct
ttcttatatataagattgctggcgcgactcacgtctaatggcaagagttgtcctccgacacagactaagaacttgttgggactgtca

SEQ ID NO: 273 - DNA, 87 bp, Artificial Sequence
  Synthetic Construct
ttcttgtcagtcttctagctaacggacgaggatcgtcgctgaccttctggtggatctttcgtcacaagagagactccgaagcgcttc

SEQ ID NO: 274 - DNA, 87 bp, Artificial Sequence
  Synthetic Construct
ttcctacctctccagaatcatctgcgactaacgggccagtctggtcaggtggtactctcgtatggccacctccgtgatgtcgtctta

SEQ ID NO: 275 - DNA, 87 bp, Artificial Sequence
  Synthetic Construct
ttcctactactataggtgcgcttcgatagcgtactcaagatactcgagcctggcaagactctgagaatctgatagagtacgggtcgt

SEQ ID NO: 276 - DNA, 87 bp, Artificial Sequence
  Synthetic Construct
ttcctgtgcggtgcttagttgtatttcaagggtggaaatacactaggcgcgttaaagctcttgagcgtaccgtctagctgaagtttc

SEQ ID NO: 277 - DNA, 87 bp, Artificial Sequence
  Synthetic Construct
ttcctgtaggtcacgggcatcttcttgactcagttgtctcagccagaggcgtcgccttgctcgacttctatagctcacttggtcata

SEQ ID NO: 278 - DNA, 87 bp, Artificial Sequence
  Synthetic Construct
ttcctactccgagagatcctacgacgacgctctcgtctgggctcgctaatccagggatcatgaccttctcgttgagagacgggagct

SEQ ID NO: 279 - DNA, 87 bp, Artificial Sequence
  Synthetic Construct
ttctaggtatatgatctaaaccattgtcagccatcgtagggtcgctagtcggcgagcaaggtatgtacaccttgcctgtctcagcag

SEQ ID NO: 280 - DNA, 87 bp, Artificial Sequence
  Synthetic Construct
ttcctatcttcttctactataagattggtctgtgcagtgaagcgcactgcacactgtagaactctcccgggatgcgtcaagcgagtc

SEQ ID NO: 281 - DNA, 87 bp, Artificial Sequence
  Synthetic Construct
ttcctgttaaattctcgaacaaagttcccgacaagactcaattcagatctccgaagaggacatataggaacattcacactcgaggac

SEQ ID NO: 282 - DNA, 87 bp, Artificial Sequence
  Synthetic Construct
ttcctgtattcggtgcagctgagacgtgcggctgatttactcgctcgatacagactagaccatctcgaggtaggatatggatagtta

SEQ ID NO: 283 - DNA, 87 bp, Artificial Sequence
  Synthetic Construct
ttcctatcgcatttacactgccagtagtcgttggctagacctacgctatcattcaagtcgagcggttagatccaggtctctccatct

SEQ ID NO: 284 - DNA, 87 bp, Artificial Sequence
  Synthetic Construct
ttctagtcacctaactgtttgacagcagcaaacacagacgcttactcgccgttcctgcagagccgcgctacagatcgttcaaagtac

SEQ ID NO: 285 - DNA, 87 bp, Artificial Sequence
  Synthetic Construct
ttcctcttcgtcccttgaggtccttgagacgtgctatgaatagatgtcacattacgagattcgagaatattggagctctctttgata

SEQ ID NO: 286 - DNA, 87 bp, Artificial Sequence
  Synthetic Construct
ttcctcttaaactgcctaaatggagtaggcgctgtgtcttatcctgatgatttggattacgaccgagacttatgatcatgcataggt

SEQ ID NO: 287 - DNA, 87 bp, Artificial Sequence
  Synthetic Construct
ttcttcggctgctctagacactgtgatgagaagcatcactgaccatagctgggaggcacggtcatcgtagagagagattcgccgcgt

SEQ ID NO: 288 - DNA, 87 bp, Artificial Sequence
  Synthetic Construct
ttctgagagttcgtcagactagtagtctgtggtgagatccagcgaaagagtcgaggcatccgtttccgatgtcgctacgagggtgtc

SEQ ID NO: 289 - DNA, 87 bp, Artificial Sequence
  Synthetic Construct
ttctgaggcaagtaggcggcgcgagcttagtgaggtctcgtacgctctagctatatgttccaggatatacagtgatcaccactcgtc

SEQ ID NO: 290 - DNA, 87 bp, Artificial Sequence
  Synthetic Construct
ttctgaggaaagaagtatttagtctatcagggcgattgatctggagatctgactgatgcagacatcggtgtcagaatattgccggga

SEQ ID NO: 291 - DNA, 87 bp, Artificial Sequence
  Synthetic Construct
ttctgagtcctgtagtgatagacttctccgttcgcatgaatgggaggcctcagagacgacctcctagacaagtgtatcatgcgagga

SEQ ID NO: 292 - DNA, 87 bp, Artificial Sequence
  Synthetic Construct
ttctgagtgtgcgagtaggtgactccttgctcgcgacgccgaactagtggaatcttcgagcatcctcgtgctgatgtcagtgtgtag

SEQ ID NO: 293 - DNA, 87 bp, Artificial Sequence
  Synthetic Construct
ttctgagcttcttgatagttctctgcagtgctgttccgcagactcgtcgctgatttcagaatcctgcctgacggattcttaagttag

SEQ ID NO: 294 - DNA, 87 bp, Artificial Sequence
  Synthetic Construct
ttctgagcgtagccgcgccctggatattgaagagtaggtgatagatatctgcgaccgacaagacgactagtcactccaaagtatcgc

SEQ ID NO: 295 - DNA, 87 bp, Artificial Sequence
  Synthetic Construct
ttctcgagctgcgatgcagctttcggtcctggacctcgacattacttcctcggcgcttgtgacggttctacgggaactccatagtgt

SEQ ID NO: 296 - DNA, 87 bp, Artificial Sequence
  Synthetic Construct
ttccctgcatcacgtttcgagcgttcatagtctggagtcgtacctcgattcaagcatatggcgtgatctctcggacagagatagaga

SEQ ID NO: 297 - DNA, 87 bp, Artificial Sequence
  Synthetic Construct
ttctcactcttcgatgagcgaagaggacctatcagaagtgaggctctaatccacctaatccctttggtatgaatcgactgcgtcggt

SEQ ID NO: 298 - DNA, 87 bp, Artificial Sequence
  Synthetic Construct
ttctcgtgagagcagaacccatcagtatctccgggcgcgcaggtggtgtagttcgcgggaggccagttctagcacctgtatccttcg

SEQ ID NO: 299 - DNA, 87 bp, Artificial Sequence
  Synthetic Construct
ttccatatagtcagttcagactaccagtgccagcgattaggactgaacagttctagatagtgcctctacctaggaacttgcatcgga

SEQ ID NO: 300 - DNA, 87 bp, Artificial Sequence
  Synthetic Construct
ttccatatctcttgacagggccagtcatgctgccgaacagcaatattgtgattcatagtgagcgtcatattcactggtaacgagcca

SEQ ID NO: 301 - DNA, 87 bp, Artificial Sequence
  Synthetic Construct
ttccatcagaatcagcgctctaagggatgccgagtgcctcgacgtctctgaaattctatgacatactctgtggactgataggtcgct

SEQ ID NO: 302 - DNA, 87 bp, Artificial Sequence
  Synthetic Construct
ttccatcaccagactccagagtgtgcgtgcgagtagcatctagacagccagcaggtacagcctcattagatggctaacaagacttgc

SEQ ID NO: 303 - DNA, 87 bp, Artificial Sequence
  Synthetic Construct
ttccatcgaactctcaaggctcacacgtgtctcaacgacttcaatctcatgatgggtcaggagcgacgctgatatcgaggtagtgtc

SEQ ID NO: 304 - DNA, 87 bp, Artificial Sequence
  Synthetic Construct
ttccaccgtatccgatgaaatggaggctgtgtctctacgaagcagcaggacagaggctctgacagaataaagttctctgatgagcct

SEQ ID NO: 305 - DNA, 87 bp, Artificial Sequence
  Synthetic Construct
ttccatctacgcccttgagagagtcgatgcatccagggtgtactggatgcaagagatagcgtcggaatcccgcgtatcataatacat

SEQ ID NO: 306 - DNA, 87 bp, Artificial Sequence
  Synthetic Construct
ttccacctcagatcatagggacgaaagtgcagctagggtcagtactcagatcgaggaatggctgatatcgtcagatctttgtacagt

SEQ ID NO: 307 - DNA, 87 bp, Artificial Sequence
  Synthetic Construct
ttccatccggtgcagtgtaatttcgagtgcggtggatctcctctaggcatggcgtagctacagttgaaggtgtcactcaattactta

SEQ ID NO: 308 - DNA, 87 bp, Artificial Sequence
  Synthetic Construct
ttctcgcagggacgaagatgacgcttagatcgagtgagaacagaggcgctcgacagatcagtcttgtacttgtcgagatctagaatc

SEQ ID NO: 309 - DNA, 87 bp, Artificial Sequence
  Synthetic Construct
ttctagtgctcaaagcctcgaagtctcggatcattggctctcgcgagctgtcagatgcacttaagtgatcgccacttagctcgtagc

SEQ ID NO: 310 - DNA, 87 bp, Artificial Sequence
  Synthetic Construct
ttctagtagatccagaacaagcctatctcggatccacgaactactgagatccagatcttgagacgtggacgcatcttctctgctctc

SEQ ID NO: 311 - DNA, 87 bp, Artificial Sequence
  Synthetic Construct
ttctagctcagaaagggtcgttagaacactcgcctgaatcctctagagtcttaggctacatagaagccaagaggcatcatcaatctc

SEQ ID NO: 312 - DNA, 87 bp, Artificial Sequence
  Synthetic Construct
ttctagtgagagggaacaaacgtcaaggtattacgtaacccaaagtcgactgctccaactacattggctggcctcatggtcgtatgc

SEQ ID NO: 313 - DNA, 87 bp, Artificial Sequence
  Synthetic Construct
ttctagcctgagttccgacctttgacgtaggatctggacatccctccttgacacagacgcgatagatagagtctatctatcaaccac

SEQ ID NO: 314 - DNA, 87 bp, Artificial Sequence
  Synthetic Construct
ttctagctaatcgtggtccgacgccgccgtgtaggatgcaacctctacgctacaggtgctggattctgatatgacgatcctacgggc

SEQ ID NO: 315 - DNA, 87 bp, Artificial Sequence
  Synthetic Construct
ttctcttctttactccagtattgatcgctcctcagagatcgatcaacgatcaagcatggactcagagaccactctgcaacactcact

SEQ ID NO: 316 - DNA, 87 bp, Artificial Sequence
  Synthetic Construct
ttctcttcaagattaggatgtatcttctgactcggagagcgagtagcgggcctcatatagtcaatgctcgcttactagaagactgac

SEQ ID NO: 317 - DNA, 87 bp, Artificial Sequence
  Synthetic Construct
ttctagcgcctcccagtagtcagttgaggcgtgagaggattctagttagtactcccttgaactatcgctactcgtgatgacgtgact

SEQ ID NO: 318 - DNA, 87 bp, Artificial Sequence
  Synthetic Construct
ttctagcaggctggtggacacaagtagcactgattcaacttgggcttcggagatggacagccaagtttcagctctcacctcccgaga

SEQ ID NO: 319 - DNA, 87 bp, Artificial Sequence
  Synthetic Construct
ttctcttgtctcataaagctcggagattgatagacgtgtgtacgatgaatacagtagaagttgtcattcatcaattcttagtgtaga

SEQ ID NO: 320 - DNA, 87 bp, Artificial Sequence
  Synthetic Construct
ttctcttgattgaagcgcgctcgcacatctgagggctcgtattatccggctgacgtcggctagggtcgcacggcaggtcaccgttgc

SEQ ID NO: 321 - DNA, 87 bp, Artificial Sequence
  Synthetic Construct
ttcttcctctgtatccagcacaagctaggatcaaactcgaatactttcctcgtccactgaggccagtcatcttcttagttatacaat

SEQ ID NO: 322 - DNA, 87 bp, Artificial Sequence
  Synthetic Construct
ttcttcctgttcgcattgctcgtgtctcgctcgctaaattgtgctacggctagagctgtgtgtagcctctagtcgctactccacact

SEQ ID NO: 323 - DNA, 87 bp, Artificial Sequence
  Synthetic Construct
ttcctctatcgacgtactttccaccctgaggtgactgacaatcagccgacattctcgggaaagtgtgcatctcagcctgcttagtta

SEQ ID NO: 324 - DNA, 87 bp, Artificial Sequence
  Synthetic Construct
ttctcaatcctcctacagtagcgaagattacaccaccattagtctcctctgtatttgagactcttcttcagcttactctgcttatct

SEQ ID NO: 325 - DNA, 87 bp, Artificial Sequence
  Synthetic Construct
ttcttctagtaggtcaatggaccttcgtcaagcctcgattcgagtactgtcagtatcactagccctgcaggagtcaatgtcgcggta

SEQ ID NO: 326 - DNA, 87 bp, Artificial Sequence
  Synthetic Construct
ttcccgggattcacttcgccaacagtatgtcattcgtaccatgcgttcgcatctggtaagaacctaactatgtaggtcgacgcatct

SEQ ID NO: 327 - DNA, 87 bp, Artificial Sequence
  Synthetic Construct
ttctctttcagtggaatcctctagctacgaccaaatggactctagaattcagcagatagtccaatccgtgatgagctacgctgagag

SEQ ID NO: 328 - DNA, 87 bp, Artificial Sequence
  Synthetic Construct
ttctagagaggtgcttgaggtcatccactaggcgacggtcagtgaactcagttcacatagagaatcctaggaccgcgccagaatcga

SEQ ID NO: 329 - DNA, 87 bp, Artificial Sequence
  Synthetic Construct
ttcttccgcgacggaaattcagatggtctgatcgtcatagtcggaggactcagttgacctacggatttgttacactaggagttgcca

SEQ ID NO: 330 - DNA, 87 bp, Artificial Sequence
  Synthetic Construct
ttcttcaacgacaatttcgtaccgtgcactcgcatgactttcgcgtgctcgttggtgctcgaggtaccgatactctgaacactcgta

SEQ ID NO: 331 - DNA, 87 bp, Artificial Sequence
  Synthetic Construct
ttcttccactagtgccagtgtctggtacagtgatgaccttgagagcattattacaagctgctccctctggtgaactgtgctgatcct

SEQ ID NO: 332 - DNA, 87 bp, Artificial Sequence
  Synthetic Construct
ttcttccagtcatagtgtatgcaggctggtgcgagcaagcatccatagcagagcttgagagctgagcctctggtggtatgcggaagt

SEQ ID NO: 333 - DNA, 87 bp, Artificial Sequence
  Synthetic Construct
ttcttcccttcgtctgtctcttcttagcgacgcctcggtcatgagatgaacctagaggacttatctcaggtgtgcagcctgctatag

SEQ ID NO: 334 - DNA, 87 bp, Artificial Sequence
  Synthetic Construct
ttcttcccggagcagactagtcgagtcccttagttcgctaagccggcaagtggaaagtagtagagaggaagaacgtcgcatctccga

SEQ ID NO: 335 - DNA, 87 bp, Artificial Sequence
  Synthetic Construct
ttcttgagatagcactgccctcgctacatcacttatactccgcgttagacgcagggtgcgagttagcattgaacgagagtatgttac

SEQ ID NO: 336 - DNA, 87 bp, Artificial Sequence
  Synthetic Construct
ttcttggtctaggagacaccttctgtactataggacctcttattgtctagcgtcggagcaaaggctacttgagctaatctcgctaca

SEQ ID NO: 337 - DNA, 87 bp, Artificial Sequence
  Synthetic Construct
ttcttggtatctacggacttcacatgtggtccgcagatctgttcttatttcttacacatcctcttcccgcctcattctagcaaccga

SEQ ID NO: 338 - DNA, 87 bp, Artificial Sequence
  Synthetic Construct
ttcttagctcagatgcgtatggctgtcgacatatcagctatggagaattgtcagttctctgcaatacctcctcgaacttagctctta

SEQ ID NO: 339 - DNA, 87 bp, Artificial Sequence
  Synthetic Construct
ttcttaacaaattgatctcattatagacgaaacgcaatcgcaccaccgtctcatagcagtcctcctacgcgaaattgcctatctcgt

SEQ ID NO: 340 - DNA, 87 bp, Artificial Sequence
  Synthetic Construct
ttcttgaactgagagatcacggagcctatggagggagatgtcacacctgtgcatcacgagaaggcgacgatactgtgaagcatacct

SEQ ID NO: 341 - DNA, 87 bp, Artificial Sequence
  Synthetic Construct
ttcttcactatattcacattagctaagcgcataatccgtggaatcatctgtttaccgtctggcttcctacaccgcgtggcggagcga

SEQ ID NO: 342 - DNA, 87 bp, Artificial Sequence
  Synthetic Construct
ttcttcacaccggtaaattacgtcatcaaccgaggatctcgcctcccattattctgaaactgagagatgggtttctcatgagcgtcg

SEQ ID NO: 343 - DNA, 87 bp, Artificial Sequence
  Synthetic Construct
ttcctgggtagcctgtgaaagcaggtacattgaaactctctcactcctcatctgccacagtgcatcaagccgggaactcgacgcata

SEQ ID NO: 344 - DNA, 87 bp, Artificial Sequence
  Synthetic Construct
ttcctgggacagaacggtctactatagctccgctgactacgtacatgtgattgaacggtacagtgactccctatgcgatataacgat

SEQ ID NO: 345 - DNA, 87 bp, Artificial Sequence
  Synthetic Construct
ttctcggtggatttcccttcgggaggaggaggacagcagctaagaacaccagcgaaggtctatggatctacaatccaggtcttccct

SEQ ID NO: 346 - DNA, 87 bp, Artificial Sequence
  Synthetic Construct
ttctcggctacgaatctatctgatatcccacacccgtacatgtctacgggatagtcagtgtgtttcaacacggcttacccaacaaag

SEQ ID NO: 347 - DNA, 87 bp, Artificial Sequence
  Synthetic Construct
ttcctgagcgtcatgactgctaagcgagtggtcccgcgacgaaatatcgagtctatctatgagctgcgagtctcagtgtgaccgcgt

SEQ ID NO: 348 - DNA, 87 bp, Artificial Sequence
  Synthetic Construct
ttcctaagatagtcgatcagatgatatcagatcacagctcactctttaagattggcgacacctttcatcatggagctgcgacgctca

SEQ ID NO: 349 - DNA, 87 bp, Artificial Sequence
  Synthetic Construct
ttcctagtcttctcgaagcctccatagggaaatggttaggcgggtgtcagattgcatgatcagatctgcagaggaggattatcaagt

SEQ ID NO: 350 - DNA, 87 bp, Artificial Sequence
  Synthetic Construct
ttcctagtgacggattcttcaagaaagcagtgaatacgacagagcgtccagtgcatgcgaagtactccggagtgttactgcgcggtc

SEQ ID NO: 351 - DNA, 87 bp, Artificial Sequence
  Synthetic Construct
ttcctggctgtacacagcctcgtgagcactacagtcgctctccgatcgcctgtaggattatatgtgtaggtaagctgttagatcgta

SEQ ID NO: 352 - DNA, 87 bp, Artificial Sequence
  Synthetic Construct
ttcctggcattaatatctgatctgcgtgagagtgcaacgccgaagggaatcatcgtctgcgatactaaggacacggtcctcagcaat

SEQ ID NO: 353 - DNA, 87 bp, Artificial Sequence
  Synthetic Construct
ttcctagacactttctcgatctattacaatgagtgcctcttcatcgcatagtatggaatagcacgtaacacactaagatatccttct

SEQ ID NO: 354 - DNA, 87 bp, Artificial Sequence
  Synthetic Construct
ttcctagaggagttcgagatacataatttcacggcgtctataggctacgaccattgttcacagcagatcgtaggcgtggcaggccgc

SEQ ID NO: 355 - DNA, 87 bp, Artificial Sequence
  Synthetic Construct
ttcccttctagccgtactccgatccagggactcaaggtcaaccctggttctctcgcgtgagtgggacgattcatgtgacactcaacg

SEQ ID NO: 356 - DNA, 87 bp, Artificial Sequence
  Synthetic Construct
ttcccttcagtctatactatgtcgtctcctgattcggaggagcatgcagatcaggagctgcctgcgtgactcgtctgacgtgtgaga

SEQ ID NO: 357 - DNA, 87 bp, Artificial Sequence
  Synthetic Construct
ttccctttctgttagcagttcatagactgatcttgcatcggagataagcatggcaagatgactggaactatatctagcaaggcgtag

SEQ ID NO: 358 - DNA, 87 bp, Artificial Sequence
  Synthetic Construct
ttccctttgcagcagacttagcgagtggtatgacagtctcatcagccatcgtctgtgtaccagcgctctcacgtgatcatcaagctg

SEQ ID NO: 359 - DNA, 87 bp, Artificial Sequence
  Synthetic Construct
ttcccttgcaaccactgatctcatatccgagtcgtacactctatgaatatactgatcgaggtcgtgcagtgaacgctcgagccattg

SEQ ID NO: 360 - DNA, 87 bp, Artificial Sequence
  Synthetic Construct
ttcccttgattgacggtcggcctctagtattcaccggcgtgcggtgagttgctatagactagaagagcgcgatcgcaggtccctagc

SEQ ID NO: 361 - DNA, 87 bp, Artificial Sequence
  Synthetic Construct
ttcccttactcttatcgaggaccgtgatagggttcatcagatagctacgcagtccctgtcgtcgatatcctctcaaatccaccgtag

SEQ ID NO: 362 - DNA, 87 bp, Artificial Sequence
  Synthetic Construct
ttcccttagcagtgacgcgaggagaacgctaatcctacgcctcgcctacatatccgatagatgagccgaggcggcctagtaggttct

SEQ ID NO: 363 - DNA, 87 bp, Artificial Sequence
  Synthetic Construct
ttcccgcagtgtttccatctcaacgtggtcccggtcaagttctagcactctcgccacacgggtctcggattcctcctaatcacattc

SEQ ID NO: 364 - DNA, 87 bp, Artificial Sequence
  Synthetic Construct
ttctagtattgaccagtctattagtgcccattcatcccagagatctaggctgtcgcgctagagctaacattgactcgcgtacgctgt

SEQ ID NO: 365 - DNA, 87 bp, Artificial Sequence
  Synthetic Construct
ttccctctcttcgatctggtacgatagcgatcaatatgtcgatagatagtagatagaatctgcgcttcgaagtcactcgatgagact

SEQ ID NO: 366 - DNA, 87 bp, Artificial Sequence
  Synthetic Construct
ttccctctaagcgtactctcttgaccgaaggtacagtctccagtgagaactggcccaggttagctcctgtcagctctaccttcatta

SEQ ID NO: 367 - DNA, 87 bp, Artificial Sequence
  Synthetic Construct
ttcccactaagaccggcgacttacctaagttatccttatctgtctgctctctacgtcttctctacaggaggtcctaataatgagaga

SEQ ID NO: 368 - DNA, 87 bp, Artificial Sequence
  Synthetic Construct
ttcttgggcagacatggaagcgcttcgtagctgaacagaccttgtttgatagtgggacctgcttagagatctatccattattgacct

SEQ ID NO: 369 - DNA, 87 bp, Artificial Sequence
  Synthetic Construct
ttcccaccgctccattcgctaccgagaaatatgcctcgctcttacgtcagaatcggagcgatagctggacgaggttgctgaggactc

SEQ ID NO: 370 - DNA, 87 bp, Artificial Sequence
  Synthetic Construct
ttctacgagactagagagccagaccctccaagctagggacctggcagagtggctctagctgatggatgtttgaattgagcgagctta

SEQ ID NO: 371 - DNA, 87 bp, Artificial Sequence
  Synthetic Construct
ttcttctgaagtacttacgctgctctcttgagcgacttcagactcctccgtcagtatagaacaactacaaatagcacgtctgtcttc

SEQ ID NO: 372 - DNA, 87 bp, Artificial Sequence
  Synthetic Construct
ttctcttactgacaggcaacgatccatgcgctctgctgtactgagggcgagggtgtccgacgtttccaggcgttcagataggtcgag

SEQ ID NO: 373 - DNA, 87 bp, Artificial Sequence
  Synthetic Construct
ttctagatggtcagtttcaaggatacgatattaataggcagctgagtaagccagcctgaccagacgatccctcgatgatattcatga

SEQ ID NO: 374 - DNA, 87 bp, Artificial Sequence
  Synthetic Construct
ttctcttagaagaagcacttctgatcgcgcgtcagaagaccaggttgtgaggcaatgcctttgatcagagagcgcaacaagatgcag

SEQ ID NO: 375 - DNA, 87 bp, Artificial Sequence
  Synthetic Construct
ttccctggatagaagcgattgctggtgacttgtcgatgatgattctagtcgggaatctgacaggtaacaagtccaatgtgtggtgga

SEQ ID NO: 376 - DNA, 87 bp, Artificial Sequence
  Synthetic Construct
ttctaccgacagactaagctgtagagcggattcaaggcactcggtgactctggattaagccgaggccgtaagtgtcagcagggactg

SEQ ID NO: 377 - DNA, 87 bp, Artificial Sequence
  Synthetic Construct
ttctagcatatagctaagggagaggtcggaggatagaacgctccgaatctccgagcacctaagtcggctaagctggctccggtaggt

SEQ ID NO: 378 - DNA, 87 bp, Artificial Sequence
  Synthetic Construct
ttctctcagtgctagaaggagtcgacaaagactcattcttgctgaagtttagctgagcagctgtgtcgaggtggaggactgaagagt

SEQ ID NO: 379 - DNA, 87 bp, Artificial Sequence
  Synthetic Construct
ttctagccaccgactcgcccgatggtatatcaggagtcagatacagtgtatgaccgacagggcctctacaagttgaacttgcagaac

SEQ ID NO: 380 - DNA, 87 bp, Artificial Sequence
  Synthetic Construct
ttcttggacgcttctagtactagttgtgctatccctagttatagccaccagcgagagtagacaggattgttaataaagaaggagcac

SEQ ID NO: 381 - DNA, 87 bp, Artificial Sequence
  Synthetic Construct
ttcttcttcttacctaacaacaagaataataataataatcctaataacaacaataacaataataacaacaacaatgattagccttga

SEQ ID NO: 382 - DNA, 87 bp, Artificial Sequence
  Synthetic Construct
ttcttgggaggagtgtcgagagagttgcgaggcagagcttgatctcattagatccatgagacgttgggactcaagtatctggagtcg

SEQ ID NO: 383 - DNA, 87 bp, Artificial Sequence
  Synthetic Construct
ttcctcagtagatacatagagagcgagtatcaggctgacggaagatgaagactatcgactgaggacgagctgggaatagcttcagtc

SEQ ID NO: 384 - DNA, 87 bp, Artificial Sequence
  Synthetic Construct
ttcttcttaaagatactaacaactgcttgcgagctggatgtcctctcgaagaattgcttcaagatcttggtgctcgagccaagccca

SEQ ID NO: 385 - DNA, 87 bp, Artificial Sequence
  Synthetic Construct
ttctagttcactactgtcatacagggctagctaataacttctcctgagtatgctcctcctggtgcttagagtgacgagacactacgt

SEQ ID NO: 386 - DNA, 87 bp, Artificial Sequence
  Synthetic Construct
ttctatggaccggctttgctctgttgatcgtcgatagacttccagctacaccacgacccgggccgaatggtattggctgatctgaag

SEQ ID NO: 387 - DNA, 87 bp, Artificial Sequence
  Synthetic Construct
ttctagtcttctatcgagtctggtcatagtcatatcgcacgaagacatggtctaagtcagcgccgaatctgtgacgtcttcttgaca

SEQ ID NO: 388 - DNA, 87 bp, Artificial Sequence
  Synthetic Construct
ttctagttaagagagtctatcatcgtcagtgtcgcgaaggatcgtcgacaccctatcaatctcgtctattctttccagcgcgtgtct

SEQ ID NO: 389 - DNA, 87 bp, Artificial Sequence
  Synthetic Construct
ttctatgacctccagtcatagcagaagtgtatcgaccatctgcctccgacaatcctcagtagacctccaccaccaatccgtgtcaga

SEQ ID NO: 390 - DNA, 87 bp, Artificial Sequence
  Synthetic Construct
ttctacgcattactggtgcacgcattccgattctacgtagtagtcagctagtctccttgccgagagaacgtccagacgtcagcactc

SEQ ID NO: 391 - DNA, 87 bp, Artificial Sequence
  Synthetic Construct
ttctcgtgcggcggatctccatagccgggtttcatgggtgtaagaggagtcggtcaggagatcttattcctcatcgcgggaagtctc

SEQ ID NO: 392 - DNA, 87 bp, Artificial Sequence
  Synthetic Construct
ttctcataggagatacgacctttcaaccgagtgctcgcgacgcacggcatccatccggtcaatacggctggtatgcagcctccactc

SEQ ID NO: 393 - DNA, 87 bp, Artificial Sequence
  Synthetic Construct
ttctcgtacggacgagctactctggctctaggagtcgatcgaaagtatacgaagaagggatgtactcagcagctcactgagcgagga

SEQ ID NO: 394 - DNA, 87 bp, Artificial Sequence
  Synthetic Construct
ttctcatcgctgtgaaactgatctctcaagtcatgagtgtacttgctccagactggatgaacaggtcagccttagtgctatatgtgc

SEQ ID NO: 395 - DNA, 87 bp, Artificial Sequence
  Synthetic Construct
ttctcatctatcctgggcccagacttcctggtccgtaagctaaattctctcttctactgagcattctatccagagttgagatctaag

SEQ ID NO: 396 - DNA, 87 bp, Artificial Sequence
  Synthetic Construct
ttctcgttgcacgtgtctatatatttcggctcatgaactctctatgtcctcctcgcggtcgtgcagctgcataagtcataggagtac

SEQ ID NO: 397 - DNA, 87 bp, Artificial Sequence
  Synthetic Construct
ttctcgttcccttactctaagtcaagtaactgattcggaccaagcttcaagcctggcccgtcaacagagccgggtaagaatgctgag

SEQ ID NO: 398 - DNA, 87 bp, Artificial Sequence
  Synthetic Construct
ttctctggagagacttagaagagtagtacgactatgacacctctgctattactcgtgacgccgcatgacgtctctggaagaccgcga

SEQ ID NO: 399 - DNA, 87 bp, Artificial Sequence
  Synthetic Construct
ttctctggtgtcggactgccgaagataccaggacagcataacttactggcgtaggacagagtccagactatcaatatccgactgcgt

SEQ ID NO: 400 - DNA, 87 bp, Artificial Sequence
  Synthetic Construct
ttctctgagatcaagctcggagtcagcatggctgtgggcccactggcttgttagagtgaccgacagagagatccacatagccctgac

SEQ ID NO: 401 - DNA, 87 bp, Artificial Sequence
  Synthetic Construct
ttcttctctttacagtcgagaacttcatcacagcctcgttagtctagttctagcgaggtatctcatagcgagctacctactggcata

SEQ ID NO: 402 - DNA, 87 bp, Artificial Sequence
  Synthetic Construct
ttcctctagatcggtcgcctcagaatccgatattatggctatcgtcatagaaaggtcgtattcactttccctcctatgagaggttac

SEQ ID NO: 403 - DNA, 87 bp, Artificial Sequence
  Synthetic Construct
ttctaggtcgtgatcgcgtctgattcacagttcttgggagctctattgggacgtaaggagctcggaaacaagcatagttgtggcatc

SEQ ID NO: 404 - DNA, 20 bp, Artificial Sequence
  Synthetic Construct
aatcttgtgggtagtaggcg

SEQ ID NO: 405 - DNA, 20 bp, Artificial Sequence
  Synthetic Construct
cctaagatgggcggaaaact

SEQ ID NO: 406 - DNA, 20 bp, Artificial Sequence
  Synthetic Construct
aatgaatgcccttccttcct

SEQ ID NO: 407 - DNA, 20 bp, Artificial Sequence
  Synthetic Construct
tcaacgtagggcgaagaaat

SEQ ID NO: 408 - DNA, 20 bp, Artificial Sequence
  Synthetic Construct
acacaataccattggcagga

SEQ ID NO: 409 - DNA, 20 bp, Artificial Sequence
  Synthetic Construct
cttgcgtgccatatctgatg

SEQ ID NO: 410 - DNA, 20 bp, Artificial Sequence
  Synthetic Construct
acagccaaagaataccgtcc

SEQ ID NO: 411 - DNA, 20 bp, Artificial Sequence
  Synthetic Construct
taagtgctcaaaacgaacgg

SEQ ID NO: 412 - DNA, 20 bp, Artificial Sequence
  Synthetic Construct
acgatggggacatagaacac

SEQ ID NO: 413 - DNA, 20 bp, Artificial Sequence
  Synthetic Construct
ttgcccttcgctcaatctag

SEQ ID NO: 414 - DNA, 20 bp, Artificial Sequence
  Synthetic Construct
acgcccactatatttcacca

SEQ ID NO: 415 - DNA, 20 bp, Artificial Sequence
  Synthetic Construct
tggggacttttaccatccag